European Patent Application EP 4 190 907 A1, published June 7, 2023. Title: Two-step method for manufacturing 3-hydroxypropionic acid. Applicant: LG CHEM, LTD. The sequence listing filed with the application follows.

SEQUENCE LISTING (6 sequences)

SEQ ID NO: 1 - DNA, 35 bp, Artificial Sequence
  dhaB-gdrA-F
gaattcatgaaaagatcaaaacgatttgcagtcct

SEQ ID NO: 2 - DNA, 29 bp, Artificial Sequence
  dhaB-gdrA-R
aagcttgatctcccactgaccaaagctgg

SEQ ID NO: 3 - DNA, 38 bp, Artificial Sequence
  gdrB-F
aagcttagagggggccgtcatgtcgctttcaccgccag

SEQ ID NO: 4 - DNA, 28 bp, Artificial Sequence
  gdrB-R
cttaagtcagtttctctcacttaacggc

SEQ ID NO: 5 - DNA, 26 bp, Artificial Sequence
  aldH-F
ggtaccatgaattttcatcatctggc

SEQ ID NO: 6 - DNA, 24 bp, Artificial Sequence
  aldH-R
catatgtcaggcctccaggcttat